European Patent Specification EP 3 628 059 B1, published April 12, 2023. Title: ASSAY FOR DETECTING HUMAN IMMUNODEFICIENCY VIRUS (HIV). Applicant: ABBOTT MOLECULAR INC. The sequence listing filed with the application follows.

SEQUENCE LISTING (54 sequences)

SEQ ID NO: 1 - DNA, 29 bp, Artificial Sequence
  Synthetic
attccctacaatccccaaagtcaaggagt

SEQ ID NO: 2 - DNA, 26 bp, Artificial Sequence
  Synthetic
ctttcccctgcactgtaccccccaat

SEQ ID NO: 3 - DNA, 43 bp, Artificial Sequence
  Synthetic
acagcagtacagatggcagtattcattcacaattttaaaagaa

SEQ ID NO: 4 - DNA, 16 bp, Artificial Sequence
  Synthetic
cggatttgtactgctg

SEQ ID NO: 5 - DNA, 27 bp, Artificial Sequence
  Synthetic
aagcctcaataaagcttgccttgagtg

SEQ ID NO: 6 - DNA, 25 bp, Artificial Sequence
  Synthetic
gtccctgttcgggcgccactgctag

SEQ ID NO: 7 - DNA, 47 bp, Artificial Sequence
  Synthetic
tgtgtgcccgtctgttgtgcgactctggtatctagagatccctcaga

SEQ ID NO: 8 - DNA, 11 bp, Artificial Sequence
  Synthetic
acgggcacaca

SEQ ID NO: 9 - DNA, 43 bp, Artificial Sequence
  Synthetic
agtgtgtgctcatctgttcaaccctggtatctagagatccctc

SEQ ID NO: 10 - DNA, 14 bp, Artificial Sequence
  Synthetic
gatgagcacacact

SEQ ID NO: 11 - DNA, 27 bp, Artificial Sequence
  Synthetic
cagagttggcagcttcactttctcttg

SEQ ID NO: 12 - DNA, 22 bp, Artificial Sequence
  Synthetic
gtctggcctttcagcaagtttc

SEQ ID NO: 13 - DNA, 24 bp, Artificial Sequence
  Synthetic
acgagttcatgagggcaggccgct

SEQ ID NO: 14 - DNA, 29 bp, Artificial Sequence
  Synthetic
attccctacaatccccaaagtcaaggagt

SEQ ID NO: 15 - DNA, 29 bp, Artificial Sequence
  Synthetic
attccctacaatccccaaagtcaaggagt

SEQ ID NO: 16 - DNA, 29 bp, Artificial Sequence
  Synthetic
attccctacaatccccaaagtcaaggagt

SEQ ID NO: 17 - DNA, 29 bp, Artificial Sequence
  Synthetic
attccctacaatccccaaagtcaaggagt

SEQ ID NO: 18 - DNA, 29 bp, Artificial Sequence
  Synthetic
attcccuacaatccccaaagtcaaggagt

SEQ ID NO: 19 - DNA, 29 bp, Artificial Sequence
  Synthetic
attcccuacaatccccaaagtcaaggagt

SEQ ID NO: 20 - DNA, 29 bp, Artificial Sequence
  Synthetic
attccctacaatccccaaagtcaaggagt

SEQ ID NO: 21 - DNA, 29 bp, Artificial Sequence
  Synthetic
attccctacaatccccaaagtcaaggagt

SEQ ID NO: 22 - DNA, 29 bp, Artificial Sequence
  Synthetic
attcccuacaatccccaaagtcaaggagt

SEQ ID NO: 23 - DNA, 28 bp, Artificial Sequence
  Synthetic
attccctacaatccccaaagtcaaggag

SEQ ID NO: 24 - DNA, 29 bp, Artificial Sequence
  Synthetic
ataccctacaatcctcaaagtcagggagc

SEQ ID NO: 25 - DNA, 27 bp, Artificial Sequence
  Synthetic
accctacaatcctcaaagtcagggagc

SEQ ID NO: 26 - DNA, 27 bp, Artificial Sequence
  Synthetic
gggataccctacaatcctcaaagtcag

SEQ ID NO: 27 - DNA, 27 bp, Artificial Sequence
  Synthetic
cgggataccctacaatcctcaaagtca

SEQ ID NO: 28 - DNA, 28 bp, Artificial Sequence
  Synthetic
cgggataccctacaatcctcaaagtcag

SEQ ID NO: 29 - DNA, 27 bp, Artificial Sequence
  Synthetic
cctacaatcctcaaagtcagggagcag

SEQ ID NO: 30 - DNA, 29 bp, Artificial Sequence
  Synthetic
gataccctacaatcctcaaagtcagggag

SEQ ID NO: 31 - DNA, 29 bp, Artificial Sequence
  Synthetic
ataccatataatccacaaagtcaaggagt

SEQ ID NO: 32 - DNA, 29 bp, Artificial Sequence
  Synthetic
ataccatataacccacaaagtcaaggagt

SEQ ID NO: 33 - DNA, 31 bp, Artificial Sequence
  Synthetic
gaataccatataatccacaaagtcaaggagt

SEQ ID NO: 34 - DNA, 31 bp, Artificial Sequence
  Synthetic
gaataccatataacccacaaagtcaaggagt

SEQ ID NO: 35 - DNA, 32 bp, Artificial Sequence
  Synthetic
ggaataccatataatccacaaagtcaaggagt

SEQ ID NO: 36 - DNA, 32 bp, Artificial Sequence
  Synthetic
ggaataccatataacccacaaagtcaaggagt

SEQ ID NO: 37 - DNA, 24 bp, Artificial Sequence
  Synthetic
ttcccctgcactgtaccccccaat

SEQ ID NO: 38 - DNA, 24 bp, Artificial Sequence
  Synthetic
tcccctgcactgtaccccccaatc

SEQ ID NO: 39 - DNA, 30 bp, Artificial Sequence
  Synthetic
gtctactattctttcccctgcactgtaccc

SEQ ID NO: 40 - DNA, 31 bp, Artificial Sequence
  Synthetic
attatgtctactattctttcccctgcactgt

SEQ ID NO: 41 - DNA, 32 bp, Artificial Sequence
  Synthetic
gtctgttgctattatgtctactattctttccc

SEQ ID NO: 42 - DNA, 29 bp, Artificial Sequence
  Synthetic
atttctgctgtccctgtaataaacccgaa

SEQ ID NO: 43 - DNA, 45 bp, Artificial Sequence
  Synthetic
gtgtgtgcccgtctgttgtgtgactctggtaactagagatccctc

SEQ ID NO: 44 - DNA, 23 bp, Artificial Sequence
  Synthetic
cugguaactagagaucccucaga

SEQ ID NO: 45 - DNA, 26 bp, Artificial Sequence
  Synthetic
actctggtaactagagatccctcaga

SEQ ID NO: 46 - DNA, 27 bp, Artificial Sequence
  Synthetic
tcagcaagccgagtcctgcgtcgagag

SEQ ID NO: 47 - DNA, 25 bp, Artificial Sequence
  Synthetic
cccgttgcgtcggaggttttcttcc

SEQ ID NO: 48 - DNA, 28 bp, Artificial Sequence
  Synthetic
aatctctagcagtggcgcccgaacaggg

SEQ ID NO: 49 - DNA, 27 bp, Artificial Sequence
  Synthetic
aatctctagcagtggcgcccgaacagg

SEQ ID NO: 50 - DNA, 27 bp, Artificial Sequence
  Synthetic
tgacgctctcgcacccatctctctcct

SEQ ID NO: 51 - DNA, 28 bp, Artificial Sequence
  Synthetic
tctctcgacgcaggactcggcttgctga

SEQ ID NO: 52 - DNA, 28 bp, Artificial Sequence
  Synthetic
aagaaaacctccgacgcaacgggctcgg

SEQ ID NO: 53 - DNA, 25 bp, Artificial Sequence
  Synthetic
ttggcagcttcactttctcttgcag

SEQ ID NO: 54 - DNA, 26 bp, Artificial Sequence
  Synthetic
agttggcagcttcactttctcttgca